European Patent Specification EP 3 669 884 B1, published October 18, 2023. Title: A composition comprising mesenchymal stem cell for treating thyroid associated ophthalmopathy. Applicant: Sungkwang medical foundation. The sequence listing filed with the application follows.

SEQUENCE LISTING (6 sequences)

SEQ ID NO: 1 - DNA, 19 bp, Artificial Sequence
  fprimer for PPAR
ttgacccagaaagcgattc

SEQ ID NO: 2 - DNA, 20 bp, Artificial Sequence
  Reverse primer for PPAR
aaagttggtgggccagaatg

SEQ ID NO: 3 - DNA, 21 bp, Artificial Sequence
  Forward primer for ADIPONECTIN
ggccgtgatgatggcagagat

SEQ ID NO: 4 - DNA, 22 bp, Artificial Sequence
  Reverse primer for ADIPONECTIN
tttcaccgatgtctcccttagg

SEQ ID NO: 5 - DNA, 20 bp, Artificial Sequence
  Forward primer for C/EBP
tgtatacccctggtgggaga

SEQ ID NO: 6 - DNA, 20 bp, Artificial Sequence
  reverse primer for C/EBP
tcataactccggtccctctg